European Patent Application EP 4 257 615 A1, published October 11, 2023. Title: SELF-ASSEMBLED NANOPARTICLE CONTAINING GB PROTEIN OF EB VIRUS AND PREPARATION METHOD AND USE THEREOF. Applicant: SUN YAT-SEN UNIVERSITY;SUN YAT-SEN UNIVERSITY CANCER CENTER(SYSUCC). The sequence listing filed with the application follows.

SEQUENCE LISTING (29 sequences)

SEQ ID NO: 1 - protein, 209 aa, Artificial Sequence
  synthesized
MKMEELFKKHKIVAVLRANSVEEAIEKAVAVFAGGVHLIEITFTVPDADTVIKALSVLKEKGAIIGAGTVTSVEQCRKAVESGAEFIVSPHLDEEISQFCKEKGVFYMPGVMTPTELVKAMKLGHDILKLFPGEVVGPQFVKAMKGPFPNVKFVPTGGVNLDNVCEWFKAGVLAVGVGDALVKGDPDEVREKAKKFVEKIRGCTEGSLE

SEQ ID NO: 2 - protein, 160 aa, Artificial Sequence
  synthesized
MNQHSHKDHETVRIAVVRARWHAEIVDACVSAFEAAMRDIGGDRFAVDVFDVPGAYEIPLHARTLAETGRYGAVLGTAFVVNGGIYRHEFVASAVINGMMNVQLNTGVPVLSAVLTPHNYDKSKAHTLLFLALFAVKGMEAARACVEILAAREKIAAGSL

SEQ ID NO: 3 - protein, 661 aa, Epstein-Barr Virus
QTPEQPAPPATTVQPTATRQQTSFPFRVCELSSHGDLFRFSSDIQCPSFGTRENHTEGLLMVFKDNIIPYSFKVRSYTKIVTNILIYNGHRADSVTNRHEEKFSVESYETDQMDTIYQCYNAVKMTKDGLTRVYVDRDGVNITVNLKPTGGLANGVRRYASQTELYDAPGRVEATYRTRTTVNCLITDMMAKSNSPFDFFVTTTGQTVEMSPFYDGKNTETFHERADSFHVRTNYKIVDYDNRGTNPQGERRAFLDKGTYTLSWKLENRTAYCPLQHWQTFDSTIATETGKSIHFVTDEGTSSFVTNTTVGIELPDAFKCIEEQVNKTMHEKYEAVQDRYTKGQEAITYFITSGGLLLAWLPLTPRSLATVKNLTELTTPTSSPPSSPSPPAPPAARGSTSAAVLRRRRRNAGNATTPVPPAAPGKSLGTLNNPATVQIQFAYDSLRRQINRMLGDLARAWCLEQKRQNMVLRELTKINPTTVMSSIYGKAVAAKRLGDVISVSQCVPVNQATVTLRKSMRVPGSETMCYSRPLVSFSFINDTKTYEGQLGTDNEIFLTKKMTEVCQATSQYYFQSGNEIHVYNDYHHFKTIELDGIATLQTFISLNTSLIENIDFASLELYSRDEQRASNVFDLEGIFREYNFQAQNIAGLRKDLDNAVS

SEQ ID NO: 4 - protein, 10 aa, Artificial Sequence
  synthesized
GGGGSGGGGS

SEQ ID NO: 5 - protein, 11 aa, Artificial Sequence
  synthesized
GGGGSGGGGSG

SEQ ID NO: 6 - protein, 12 aa, Artificial Sequence
  synthesized
GGGGSGGGGSGS

SEQ ID NO: 7 - protein, 13 aa, Artificial Sequence
  synthesized
GGGGSGGGGSGGS

SEQ ID NO: 8 - protein, 14 aa, Artificial Sequence
  synthesized
GGGGSGGGGSGGGS

SEQ ID NO: 9 - protein, 15 aa, Artificial Sequence
  synthesized
GGGGSGGGGSGGGGS

SEQ ID NO: 10 - protein, 27 aa, Artificial Sequence
  synthesized
GYIPEAPRDGQAYVRKDGEWVLLSTFL

SEQ ID NO: 11 - protein, 32 aa, Artificial Sequence
  synthesized
MKQIEDKIEEILSKIYHIENEIARIKKLIGEV

SEQ ID NO: 12 - DNA, 1983 bp, Epstein-Barr Virus
cagaccccagagcagcctgcaccacctgccaccacagtgcagcctacagccaccagacagcagaccagcttccccttccgggtgtgcgagctgagctcccacggcgacctgttcagattttctagcgatatccagtgtccctccttcggcacaagggagaaccacaccgagggcctgctgatggtgttcaaggacaatatcatcccttactcctttaaggtgagatcttatacaaagatcgtgaccaacatcctgatctacaatggccacagagccgattctgtgaccaacaggcacgaggagaagtttagcgtggagtcctatgagacagaccagatggataccatctaccagtgctataatgccgtgaagatgacaaaggacggcctgaccagagtgtacgtggacagggatggcgtgaacatcacagtgaatctgaagcctaccggaggactggcaaacggcgtgcggagatacgccagccagaccgagctgtatgatgcaccaggaagggtggaggcaacatacaggaccaggaccacagtgaactgtctgatcacagacatgatggccaagagcaattccccattcgatttctttgtgaccacaaccggccagaccgtggagatgagccccttttatgacggcaagaacacagagaccttccacgagcgcgccgattcctttcacgtgcggacaaattacaagatcgtggactatgataacagaggaaccaatccacagggagagaggagggccttcctggacaagggcacatacaccctgtcctggaagctggagaacaggacagcctattgccccctgcagcactggcagacatttgactccaccatcgccacagagaccggcaagtctatccacttcgtgacagatgagggcacctcctcttttgtgaccaacacaaccgtgggcatcgagctgcccgacgccttcaagtgtatcgaggagcaagtgaataagacaatgcacgagaagtacgaggccgtgcaggatcgctataccaagggccaggaagccatcacatactttatcaccagcggaggactgctgctggcatggctgccactgacaccacggtccctggccacagtgaagaatctgaccgagctgacaaccccaaccagctccccaccatctagcccaagccctccagcaccacctgcagcacggggctctaccagcgccgccgtgctgcggagaaggcgccggaacgcaggaaatgcaacaacccctgtgccaccagcagcacctggcaagtctctgggcacactgaacaatcccgccaccgtgcagatccagttcgcctacgacagcctgagaaggcagatcaacagaatgctgggcgatctggcaagggcatggtgcctggagcagaagcgccagaacatggtgctgcgggagctgaccaagatcaatcctacaaccgtgatgtcctctatctatggcaaggcagtggcagcaaagagactgggcgacgtgatctccgtgtctcagtgcgtgccagtgaatcaggccacagtgaccctgagaaagagcatgagggtgcccggctccgagaccatgtgctactctaggcctctggtgagcttctcctttatcaacgacacaaagacctatgagggccagctgggcacagataatgagatcttcctgacaaagaagatgaccgaggtgtgccaggccaccagccagtactatttccagtccggcaacgagatccacgtgtacaatgactatcaccactttaagacaatcgagctggatggcatcgccacactgcagaccttcatctctctgaacaccagcctgatcgagaatatcgactttgccagcctggagctgtactccagggacgagcagagggcatccaacgtgttcgatctggagggcatcttccgcgagtataactttcaggcccagaatatcgccggcctgcggaaggacctggataatgccgtgtct

SEQ ID NO: 13 - DNA, 30 bp, Artificial Sequence
  synthesized
ggaggaggaggaagcggaggaggaggatcc

SEQ ID NO: 14 - DNA, 33 bp, Artificial Sequence
  synthesized
ggaggaggaggaagcggaggaggaggatccggc

SEQ ID NO: 15 - DNA, 36 bp, Artificial Sequence
  synthesized
ggaggaggaggaagcggaggaggaggatccggcggc

SEQ ID NO: 16 - DNA, 39 bp, Artificial Sequence
  synthesized
ggaggaggaggaagcggaggaggaggatccggcggcggc

SEQ ID NO: 17 - DNA, 42 bp, Artificial Sequence
  synthesized
ggaggaggaggaagcggaggaggaggatccggcggcggcggc

SEQ ID NO: 18 - DNA, 45 bp, Artificial Sequence
  synthesized
ggaggaggaggaagcggaggaggaggatccggcggcggcggctct

SEQ ID NO: 19 - DNA, 81 bp, Artificial Sequence
  synthesized
ggatacatccctgaggcaccaagggacggacaggcctatgtgcggaaggatggcgagtgggtgctgctgtccaccttcctg

SEQ ID NO: 20 - DNA, 627 bp, Artificial Sequence
  synthesized
atgaagatggaggagctgtttaagaagcacaagatcgtggccgtgctgagggccaactccgtggaggaggccatcgagaaggcagtggccgtgttcgcaggaggagtgcacctgatcgagatcaccttcaccgtgccagacgccgataccgtgatcaaggccctgtccgtgctgaaggagaagggagcaatcatcggagcaggaacagtgacctctgtggagcagtgcaggaaggcagtggagtctggagccgagttcatcgtgagccctcacctggacgaggagatcagccagttctgtaaggagaagggcgtgttttacatgcccggcgtgatgacacctaccgagctggtgaaggccatgaagctgggccacgatatcctgaagctgttcccaggagaggtggtgggacctcagtttgtgaaggccatgaagggccctttcccaaacgtgaagtttgtgcccacaggcggcgtgaacctggacaacgtgtgcgagtggttcaaggcaggcgtgctggcagtgggagtgggcgatgccctggtgaagggcgaccctgatgaggtgcgcgagaaggccaagaagtttgtggagaagatcaggggatgtaccgagggcagcctggag

SEQ ID NO: 21 - DNA, 72 bp, Artificial Sequence
  synthesized
atgccaatgggctctctgcagcccctggccacactgtacctgctgggaatgctggtggcaagctgcctggga

SEQ ID NO: 22 - DNA, 24 bp, Artificial Sequence
  synthesized
catcatcaccaccaccaccaccac

SEQ ID NO: 23 - DNA, 483 bp, Artificial Sequence
  synthesized
atgaaccagcacagccacaaggaccacgagaccgtgcgtattgcggtggttcgtgcgcgttggcatgcggagattgtggatgcgtgcgttagcgcgttcgaagcggcgatgcgtgacatcggtggcgatcgtttcgcggtggacgtttttgatgtgccgggtgcgtacgagattccgctgcatgcgcgtaccctggcggaaaccggtcgttatggcgcggttctgggcaccgcgttcgtggttaacggtggcatctaccgtcacgaatttgtggcgagcgcggttattaacggtatgatgaacgtgcaactgaacaccggcgtgccggttctgagcgcggttctgaccccgcacaactatgacaagagcaaagcgcacaccctgctgttcctggcgctgtttgcggtgaagggtatggaagcggcgcgtgcgtgcgttgagatcctggcggcgcgtgaaaaaattgcggcgggcagcctggaa

SEQ ID NO: 24 - DNA, 18 bp, Artificial Sequence
  synthesized
catcatcaccaccaccac

SEQ ID NO: 25 - protein, 24 aa, Artificial Sequence
  synthesized
MPMGSLQPLATLYLLGMLVASCLG

SEQ ID NO: 26 - DNA, 12 bp, Artificial Sequence
  synthesized
caccaccaccac

SEQ ID NO: 27 - DNA, 2844 bp, Artificial Sequence
  synthesized
atgccaatgggctctctgcagcccctggccacactgtacctgctgggaatgctggtggcaagctgcctgggacagaccccagagcagcctgcaccacctgccaccacagtgcagcctacagccaccagacagcagaccagcttccccttccgggtgtgcgagctgagctcccacggcgacctgttcagattttctagcgatatccagtgtccctccttcggcacaagggagaaccacaccgagggcctgctgatggtgttcaaggacaatatcatcccttactcctttaaggtgagatcttatacaaagatcgtgaccaacatcctgatctacaatggccacagagccgattctgtgaccaacaggcacgaggagaagtttagcgtggagtcctatgagacagaccagatggataccatctaccagtgctataatgccgtgaagatgacaaaggacggcctgaccagagtgtacgtggacagggatggcgtgaacatcacagtgaatctgaagcctaccggaggactggcaaacggcgtgcggagatacgccagccagaccgagctgtatgatgcaccaggaagggtggaggcaacatacaggaccaggaccacagtgaactgtctgatcacagacatgatggccaagagcaattccccattcgatttctttgtgaccacaaccggccagaccgtggagatgagccccttttatgacggcaagaacacagagaccttccacgagcgcgccgattcctttcacgtgcggacaaattacaagatcgtggactatgataacagaggaaccaatccacagggagagaggagggccttcctggacaagggcacatacaccctgtcctggaagctggagaacaggacagcctattgccccctgcagcactggcagacatttgactccaccatcgccacagagaccggcaagtctatccacttcgtgacagatgagggcacctcctcttttgtgaccaacacaaccgtgggcatcgagctgcccgacgccttcaagtgtatcgaggagcaagtgaataagacaatgcacgagaagtacgaggccgtgcaggatcgctataccaagggccaggaagccatcacatactttatcaccagcggaggactgctgctggcatggctgccactgacaccacggtccctggccacagtgaagaatctgaccgagctgacaaccccaaccagctccccaccatctagcccaagccctccagcaccacctgcagcacggggctctaccagcgccgccgtgctgcggagaaggcgccggaacgcaggaaatgcaacaacccctgtgccaccagcagcacctggcaagtctctgggcacactgaacaatcccgccaccgtgcagatccagttcgcctacgacagcctgagaaggcagatcaacagaatgctgggcgatctggcaagggcatggtgcctggagcagaagcgccagaacatggtgctgcgggagctgaccaagatcaatcctacaaccgtgatgtcctctatctatggcaaggcagtggcagcaaagagactgggcgacgtgatctccgtgtctcagtgcgtgccagtgaatcaggccacagtgaccctgagaaagagcatgagggtgcccggctccgagaccatgtgctactctaggcctctggtgagcttctcctttatcaacgacacaaagacctatgagggccagctgggcacagataatgagatcttcctgacaaagaagatgaccgaggtgtgccaggccaccagccagtactatttccagtccggcaacgagatccacgtgtacaatgactatcaccactttaagacaatcgagctggatggcatcgccacactgcagaccttcatctctctgaacaccagcctgatcgagaatatcgactttgccagcctggagctgtactccagggacgagcagagggcatccaacgtgttcgatctggagggcatcttccgcgagtataactttcaggcccagaatatcgccggcctgcggaaggacctggataatgccgtgtctggaggaggaggaagcggaggaggaggatccggcggcggcggctctggatacatccctgaggcaccaagggacggacaggcctatgtgcggaaggatggcgagtgggtgctgctgtccaccttcctgggctctggcagccatcatcaccaccaccaccaccacatgaagatggaggagctgtttaagaagcacaagatcgtggccgtgctgagggccaactccgtggaggaggccatcgagaaggcagtggccgtgttcgcaggaggagtgcacctgatcgagatcaccttcaccgtgccagacgccgataccgtgatcaaggccctgtccgtgctgaaggagaagggagcaatcatcggagcaggaacagtgacctctgtggagcagtgcaggaaggcagtggagtctggagccgagttcatcgtgagccctcacctggacgaggagatcagccagttctgtaaggagaagggcgtgttttacatgcccggcgtgatgacacctaccgagctggtgaaggccatgaagctgggccacgatatcctgaagctgttcccaggagaggtggtgggacctcagtttgtgaaggccatgaagggccctttcccaaacgtgaagtttgtgcccacaggcggcgtgaacctggacaacgtgtgcgagtggttcaaggcaggcgtgctggcagtgggagtgggcgatgccctggtgaagggcgaccctgatgaggtgcgcgagaaggccaagaagtttgtggagaagatcaggggatgtaccgagggcagcctggag

SEQ ID NO: 28 - protein, 948 aa, Artificial Sequence
  synthesized
MPMGSLQPLATLYLLGMLVASCLGQTPEQPAPPATTVQPTATRQQTSFPFRVCELSSHGDLFRFSSDIQCPSFGTRENHTEGLLMVFKDNIIPYSFKVRSYTKIVTNILIYNGHRADSVTNRHEEKFSVESYETDQMDTIYQCYNAVKMTKDGLTRVYVDRDGVNITVNLKPTGGLANGVRRYASQTELYDAPGRVEATYRTRTTVNCLITDMMAKSNSPFDFFVTTTGQTVEMSPFYDGKNTETFHERADSFHVRTNYKIVDYDNRGTNPQGERRAFLDKGTYTLSWKLENRTAYCPLQHWQTFDSTIATETGKSIHFVTDEGTSSFVTNTTVGIELPDAFKCIEEQVNKTMHEKYEAVQDRYTKGQEAITYFITSGGLLLAWLPLTPRSLATVKNLTELTTPTSSPPSSPSPPAPPAARGSTSAAVLRRRRRNAGNATTPVPPAAPGKSLGTLNNPATVQIQFAYDSLRRQINRMLGDLARAWCLEQKRQNMVLRELTKINPTTVMSSIYGKAVAAKRLGDVISVSQCVPVNQATVTLRKSMRVPGSETMCYSRPLVSFSFINDTKTYEGQLGTDNEIFLTKKMTEVCQATSQYYFQSGNEIHVYNDYHHFKTIELDGIATLQTFISLNTSLIENIDFASLELYSRDEQRASNVFDLEGIFREYNFQAQNIAGLRKDLDNAVSGGGGSGGGGSGGGGSGYIPEAPRDGQAYVRKDGEWVLLSTFLGSGSHHHHHHHHMKMEELFKKHKIVAVLRANSVEEAIEKAVAVFAGGVHLIEITFTVPDADTVIKALSVLKEKGAIIGAGTVTSVEQCRKAVESGAEFIVSPHLDEEISQFCKEKGVFYMPGVMTPTELVKAMKLGHDILKLFPGEVVGPQFVKAMKGPFPNVKFVPTGGVNLDNVCEWFKAGVLAVGVGDALVKGDPDEVREKAKKFVEKIRGCTEGSLE

SEQ ID NO: 29 - protein, 167 aa, Artificial Sequence
  synthesized
MNQHSHKDHETVRIAVVRARWHAEIVDACVSAFEAAMRDIGGDRFAVDVFDVPGAYEIPLHARTLAETGRYGAVLGTAFVVNGGIYRHEFVASAVINGMMNVQLNTGVPVLSAVLTPHNYDKSKAHTLLFLALFAVKGMEAARACVEILAAREKIAAGSLEHHHHHH